European Patent Application EP 4 190 802 A1, published June 7, 2023. Title: Cell-penetrating peptide and use thereof. Applicant: YANG SHENG TANG COMPANY, LTD.; XIAMEN UNIVERSITY. The sequence listing filed with the application follows.

SEQUENCE LISTING (54 sequences)

SEQ ID NO: 1 - protein, 239 aa, Artificial Sequence
  Amino acid sequence of GFP
MVSKGEELFTGVVPILVELDGDVNGHKFSVSGEGEGDATYGKLTLKFICTTGKLPVPWPTLVTTLTYGVQCFSRYPDHMKQHDFFKSAMPEGYVQERTIFFKDDGNYKTRAEVKFEGDTLVNRIELKGIDFKEDGNILGHKLEYNYNSHNVYIMADKQKNGIKVNFKIRHNIEDGSVQLADHYQQNTPIGDGPVLLPDNHYLSTQSALSKDPNEKRDHMVLLEFVTAAGITLGMDELYK

SEQ ID NO: 2 - protein, 147 aa, Artificial Sequence
  Amino acid sequence of DNA-binding domain of Gal4
MKLLSSIEQACDICRLKKLKCSKEKPKCAKCLKNNWECRYSPKTKRSPLTRAHLTEVESRLERLEQLFLLIFPREDLDMILKMDSLQDIKALLTGLFVQDNVNKDAVTDRLASVETDMPLTLRQHRISATSSSEESSNKGQRQLTVS

SEQ ID NO: 3 - protein, 130 aa, Artificial Sequence
  Amino acid sequence of Anti-GFP VHH2
MADVQLQESGGGSVQAGEALRLSCVGSGYTSINPYMAWFRQAPGKEREGVAAISSGGQYTYYADSVKGRFTISRDNAKNTMYLQMPSLKPDDSAKYYCAADFRRGGSWNVDPLRYDYQHWGQGTQVTVSS

SEQ ID NO: 4 - protein, 78 aa, Artificial Sequence
  Amino acid sequence of VP16 activation domain
APPTDVSLGDELHLDGEDVAMAHADALDDFDLDMLGDGDSPGPGFTPHDSAPYGALDMADFEFEQMFTDALGIDEYGG

SEQ ID NO: 5 - protein, 128 aa, Artificial Sequence
  Amino acid sequence of Anti-GFP VHH6
MADVQLQESGGGSVQTGGSLRLSCAVSPYIGSRISLGWFRQAPGKVREGVALINSRDGSTYYADTVKGRFTISQGDANTVYLQMNSLKPEDTAIYYCAARWGQITDIQALAVASFPDWGQGTQVTVSS

SEQ ID NO: 6 - protein, 236 aa, Artificial Sequence
  Amino acid sequence of RFP
MVSKGEEDNMAIIKEFMRFKVHMEGSVNGHEFEIEGEGEGRPYEGTQTAKLKVTKGGPLPFAWDILSPQFMYGSKAYVKHPADIPDYLKLSFPEGFKWERVMNFEDGGVVTVTQDSSLQDGEFIYKVKLRGTNFPSDGPVMQKKTMGWEASSERMYPEDGALKGEIKQRLKLKDGGHYDAEVKTTYKAKKPVQLPGAYNVNIKLDITSHNEDYTIVEQYERAEGRHSTGGMDGCTS

SEQ ID NO: 7 - protein, 185 aa, Artificial Sequence
  Amino acid sequence of luciferase
MGVKVLFALICIAVAEAKPTENNEDFNIVAVASNFATTDLDADRGKLPGKKLPLEVLKELEANARKAGCTRGCLICLSHIKCTPKMKKFIPGRCHTYEGDKESAQGGIGEAIVDIPEIPGFKDLEPLEQFIAQVDLCVDCTTGCLKGLANVQCSDLLKKWLPQRCATFASKIQGQVDKIKGAGGD

SEQ ID NO: 8 - DNA, 358 bp, Artificial Sequence
  UAS sequence
agcttgcatgcctgcaggtcggagtactgtcctccgagcggagtactgtcctccgagcggagtactgtcctccgagcggagtactgtcctccgagcggagtactgtcctccgagcggagactctagcgagcgccggagtataaatagaggcgcttcgtctacggagcgacaattcaattcaaacaagcaaagtgaacacgtcgctaagcgaaagctaagcaaataaacaagcgcagctgaacaagctaaacaatctgcagtaaagtgcaagttaaagtgaatcaattaaaagtaaccagcaaccaagtaaatcaactgcaactactgaaatctgccaagaagtaattattgaatacaa

SEQ ID NO: 9 - protein, 311 aa, Artificial Sequence
  Amino acid sequence of iRFP670
MARKVDLTSCDREPIHIPGSIQPCGCLLACDAQAVRITRITENAGAFFGRETPRVGELLADYFGETEAHALRNALAQSSDPKRPALIFGWRDGLTGRTFDISLHRHDGTSIIEFEPAAAEQADNPLRLTRQIIARTKELKSLEEMAARVPRYLQAMLGYHRVMLYRFADDGSGMVIGEAKRSDLESFLGQHFPASLVPQQARLLYLKNAIRVVSDSRGISSRIVPEHDASGAALDLSFAHLRSISPCHLEFLRNMGVSASMSLSIIIDGTLWGLIICHHYEPRAVPMAQRVAAEMFADFLSLHFTAAHHQR

SEQ ID NO: 10 - protein, 34 aa, Artificial Sequence
  Amino acid sequence of cpp28
RRRGRSPRRRTPSPRRRRSQSPRRRRSQSRESQC

SEQ ID NO: 11 - protein, 32 aa, Artificial Sequence
  Amino acid sequence of cpp28a
RRRGRSPRRRTPSPRRRRSQSPRRRRSQSRES

SEQ ID NO: 12 - protein, 29 aa, Artificial Sequence
  Amino acid sequence of cpp28b
RRRGRSPRRRTPSPRRRRSQSPRRRRSQS

SEQ ID NO: 13 - protein, 27 aa, Artificial Sequence
  Amino acid sequence of cpp28c
RRRGRSPRRRTPSPRRRRSQSPRRRRS

SEQ ID NO: 14 - protein, 21 aa, Artificial Sequence
  Amino acid sequence of cpp28d
RRRGRSPRRRTPSPRRRRSQS

SEQ ID NO: 15 - protein, 36 aa, Artificial Sequence
  Amino acid sequence of cpp28e
RRRDRGRSPRRRTPSPRRRRSQSPRRRRSQSRESQC

SEQ ID NO: 16 - protein, 34 aa, Artificial Sequence
  Amino acid sequence of cpp28f
RRRGRSPRRRTPSPRRRRSKSPRRRRSKSRESQC

SEQ ID NO: 17 - protein, 34 aa, Artificial Sequence
  Amino acid sequence of cpp28g
RQRGRAPRRRTPSPRRRRSQSPRRRRSQSRASQC

SEQ ID NO: 18 - protein, 37 aa, Artificial Sequence
  Amino acid sequence of cpp28h
RCRGRRGRSPRRRTPSPRRRRSQSPRRRRSKSRESQC

SEQ ID NO: 19 - protein, 39 aa, Artificial Sequence
  Amino acid sequence of cpp28i
RRRGGARASRSPRRRTPSPRRRRSQSPRRRRSQSRSANC

SEQ ID NO: 20 - protein, 40 aa, Artificial Sequence
  The amino acid sequence of cpp28j
RRRGNPRAPRSPRRRTPSPRRRRSQSPRRRRSQSPAPSNC

SEQ ID NO: 21 - protein, 40 aa, Artificial Sequence
  Amino acid sequence of cpp28k
RRRGGSRATRSPRRRTPSPRRRRSQSPRRRRSQSPASSNC

SEQ ID NO: 22 - protein, 35 aa, Artificial Sequence
  The amino acid sequence of cpp28L
RRRPASRRSTPSPRRRRSQSPRRRRSPSPRPASNC

SEQ ID NO: 23 - protein, 34 aa, Artificial Sequence
  The amino acid sequence of cpp28-Os
RRRGRSPRRRTPSPRRRRSQSPRRRRSQSRESQS

SEQ ID NO: 24 - protein, 32 aa, Artificial Sequence
  Amino acid sequence of cpp28aC
RRRGRSPRRRTPSPRRRRSQSPRRRRSQSREC

SEQ ID NO: 25 - protein, 29 aa, Artificial Sequence
  Amino acid sequence of cpp28bC
RRRGRSPRRRTPSPRRRRSQSPRRRRSQC

SEQ ID NO: 26 - protein, 27 aa, Artificial Sequence
  The amino acid sequence of cpp28cC
RRRGRSPRRRTPSPRRRRSQSPRRRRC

SEQ ID NO: 27 - protein, 21 aa, Artificial Sequence
  Amino acid sequence of cpp28dC
RRRGRSPRRRTPSPRRRRSQC

SEQ ID NO: 28 - protein, 24 aa, Artificial Sequence
  Amino acid sequence of cpp28dREC
RRRGRSPRRRTPSPRRRRSQRREC

SEQ ID NO: 29 - protein, 29 aa, Artificial Sequence
  Amino acid sequence of cpp28oNT-1
SPRRRTPSPRRRRSQSPRRRRSQSRESQC

SEQ ID NO: 30 - protein, 22 aa, Artificial Sequence
  The amino acid sequence of cpp28oNT-2
SPRRRRSQSPRRRRSQSRESQC

SEQ ID NO: 31 - protein, 14 aa, Artificial Sequence
  Amino acid sequence of cpp28oNT-3
SPRRRRSQSRESQC

SEQ ID NO: 32 - protein, 32 aa, Artificial Sequence
  Amino acid sequence of cpp28aCQ1
RRRGRQPRRRTPSPRRRRSQSPRRRRSQSREC

SEQ ID NO: 33 - protein, 32 aa, Artificial Sequence
  Amino acid sequence of cpp28aCQ2
RRRGRQPRRRTPQPRRRRSQSPRRRRSQSREC

SEQ ID NO: 34 - protein, 32 aa, Artificial Sequence
  The amino acid sequence of cpp28aCQ3
RRRGRQPRRRTPQPRRRRSQQPRRRRSQSREC

SEQ ID NO: 35 - protein, 27 aa, Artificial Sequence
  Amino acid sequence of cpp28aCNT
SPRRRTPSPRRRRSQSPRRRRSQSREC

SEQ ID NO: 36 - protein, 24 aa, Artificial Sequence
  Amino acid sequence of cpp28bCNT
SPRRRTPSPRRRRSQSPRRRRSQC

SEQ ID NO: 37 - protein, 22 aa, Artificial Sequence
  Amino acid sequence of cpp28cCNT
SPRRRTPSPRRRRSQSPRRRRC

SEQ ID NO: 38 - protein, 16 aa, Artificial Sequence
  Amino acid sequence of cpp28dCNT
SPRRRTPSPRRRRSQC

SEQ ID NO: 39 - protein, 15 aa, Artificial Sequence
  Amino acid sequence of flexible peptide linker
GGGGSGGGGSGGGGS

SEQ ID NO: 40 - protein, 288 aa, Artificial Sequence
  Amino acid sequence of GFP-cpp28
MVSKGEELFTGVVPILVELDGDVNGHKFSVSGEGEGDATYGKLTLKFICTTGKLPVPWPTLVTTLTYGVQCFSRYPDHMKQHDFFKSAMPEGYVQERTIFFKDDGNYKTRAEVKFEGDTLVNRIELKGIDFKEDGNILGHKLEYNYNSHNVYIMADKQKNGIKVNFKIRHNIEDGSVQLADHYQQNTPIGDGPVLLPDNHYLSTQSALSKDPNEKRDHMVLLEFVTAAGITLGMDELYKGGGGSGGGGSGGGGSRRRGRSPRRRTPSPRRRRSQSPRRRRSQSRESQC

SEQ ID NO: 41 - protein, 267 aa, Artificial Sequence
  Amino acid sequence of GFP-TAT
MVSKGEELFTGVVPILVELDGDVNGHKFSVSGEGEGDATYGKLTLKFICTTGKLPVPWPTLVTTLTYGVQCFSRYPDHMKQHDFFKSAMPEGYVQERTIFFKDDGNYKTRAEVKFEGDTLVNRIELKGIDFKEDGNILGHKLEYNYNSHNVYIMADKQKNGIKVNFKIRHNIEDGSVQLADHYQQNTPIGDGPVLLPDNHYLSTQSALSKDPNEKRDHMVLLEFVTAAGITLGMDELYKGGGGSGGGGSGGGGSGRKKRRQRRRPPQ

SEQ ID NO: 42 - protein, 13 aa, Artificial Sequence
  Amino acid sequence of cell-penetrating peptide TAT
GRKKRRQRRRPPQ

SEQ ID NO: 43 - protein, 237 aa, Artificial Sequence
  Amino acid sequence of mRuby3 protein
MVSKGEELIKENMRMKVVMEGSVNGHQFKCTGEGEGRPYEGVQTMRIKVIEGGPLPFAFDILATSFMYGSRTFIKYPADIPDFFKQSFPEGFTWERVTRYEDGGVVTVTQDTSLEDGELVYNVKVRGVNFPSNGPVMQKKTKGWEPNTEMMYPADGGLRGYTDIALKVDGGGHLHCNFVTTYRSKKTVGNIKMPGVHAVDHRLERIEESDNETYVVQREVAVAKYSNLGGGMDELYK

SEQ ID NO: 44 - protein, 87 aa, Artificial Sequence
  Amino acid sequence of anti-CRISPR protein
MNINDLIREIKNKDYTVKLSGTDSNSITQLIIRVNNDGNEYVISESENESIVEKFISAFKNGWNQEYEDEEEFYNDMQTITLKSELN

SEQ ID NO: 45 - protein, 136 aa, Artificial Sequence
  Amino acid sequence of anti-CRISPR-cpp28ori protein
MNINDLIREIKNKDYTVKLSGTDSNSITQLIIRVNNDGNEYVISESENESIVEKFISAFKNGWNQEYEDEEEFYNDMQTITLKSELNGGGGSGGGGSGGGGSRRRGRSPRRRTPSPRRRRSQSPRRRRSQSRESQC

SEQ ID NO: 46 - protein, 1368 aa, Artificial Sequence [sequence omitted]

SEQ ID NO: 47 - protein, 107 aa, Artificial Sequence
  Amino acid sequence of light chain variable region of antibody 2A7
DIQMTQTSSSLSASPGDRVTISCRASQGINNYLNWYKQKTDGTFKLLIYYTSYLHSGVPSRFSGRGSGTDYSLTISNLEPEDVATYYCQQYGKLPWTFGGGTKLEIK

SEQ ID NO: 48 - protein, 122 aa, Artificial Sequence
  Amino acid sequence of heavy chain variable region of antibody 2A7
QVQLQQPGAELVKPGASVKLSCKASGYTFTRYWMHWVMQRPGQDLEWIGEINPINGRTNYNEKFRRKATLTVDKSSSTVYIQFSSLTSEDSAVYFCTREGYRNDYYYAMDFWGRGTSVTVSS

SEQ ID NO: 49 - protein, 111 aa, Artificial Sequence
  Amino acid sequence of light chain variable region of antibody 16D5
DIVLTQSPGSLAVFLGQRATISCRASQSVSGSIYSYMHWYQQKPGQPPKLLIKFASNLESGVPARFSGGGSGTDFTLNIHPVEEEDAATYYCQHSWEIPYTFGGGTKLEIK

SEQ ID NO: 50 - protein, 121 aa, Artificial Sequence
  Amino acid sequence of heavy chain variable region of antibody 16D5
EVQLQQSGAEVVKPGASVKLSCTASGFKIEDTYIHWVKQRPEQGLEWIGRIDPANGNSRYDPNFQGKATIIADTSSYTIYLQLSSLTSEDTAVYYCSSPLSLLRLGGFAYWGQGTLITVSA

SEQ ID NO: 51 - protein, 107 aa, Artificial Sequence
  Amino acid sequence of light chain variable region of antibody TA99
AIQMSQSPASLSASVGETVTITCRASGNIYNYLAWYQQKQGKSPHLLVYDAKTLADGVPSRFSGSGSGTQYSLKISSLQTEDSGNYYCQHFWSLPFTFGSGTKLEIK

SEQ ID NO: 52 - protein, 120 aa, Artificial Sequence
  Amino acid sequence of heavy chain variable region of antibody TA99
VQLQQSGAELVRPGALVKLSCKTSGFNIKDYFLHWVRQRPDQGLEWIGWINPDNGNTVYDPKFQGTASLTADTSSNTVYLQLSGLTSEDTAVYFCTRRDYTYEKAALDYWGQGASVIVSS

SEQ ID NO: 53 - protein, 91 aa, Artificial Sequence
  Amino acid sequence of ZF protein
VSRPGERPFQCRICMRNFSDKTKLRVHTRTHTGEKPFQCRICMRNFSVRHNLTRHLRTHTGEKPFQCRICMRNFSQSTSLQRHLKTHLRGS

SEQ ID NO: 54 - DNA, 11 bp, Artificial Sequence
  Binding sequence of ZF protein
tgtagatggag